European Patent Application EP 4 480 497 A1, published December 25, 2024. Title: Bio-Conjugates for Oncology. Applicant: RDP Pharma AG. Application EP. The sequence listing filed with the application follows.

SEQUENCE LISTING (95 sequences)

SEQ ID NO: 1 - protein, 19 aa, synthetic construct
  REGION 1..19: note = peptide
  SITE 1: note = Variant - X0, is present or not, and if present, is an amino acid linker
  SITE 3: note = Variant - X1, is N or S, wherein N is asparagine and S is serine
  SITE 4: note = Variant - X2, is S or T, wherein S is serine and T is threonine
  SITE 6: note = Variant - X3, is present or not and, if present, is S, wherein S is serine
  SITE 7: note = Variant - X4, is present or not and, if present, is G, wherein G is glycine
  SITE 8: note = Variant - X5, is a basic polypeptide stretch consisting of 5 basic amino acid residues selected from R and K, wherein R is arginine and K is lysine, preferably wherein X5 comprises at least 3 K amino acid residues, especially wherein X5 is KKKKK or KRKKK
  SITE 10: note = Variant - X6, is a basic amino acid residue selected from R and K, wherein R is arginine and K is lysine, preferably wherein X6 is K
  SITE 11: note = Variant - X7, is S or L, wherein S is serine and L is leucine
  SITE 12: note = Variant - X8, is present or not and, if present, is a polypeptide stretch consisting of the amino acid sequence GLGS, wherein G is glycine, L is leucine and S is serine
  SITE 14: note = Variant - X9, is a basic polypeptide stretch consisting of 3 basic amino acid residues selected from R and K, wherein R is arginine and K is lysine, preferably wherein X9 comprises at least 2 K amino acid residues, especially wherein X9 is KKK or KKR
  SITE 15: note = Variant - X10, is present or not and, if present, is L or a polypeptide stretch consisting of the amino acid sequence DPL or DPC, wherein L is leucine, D is aspartic acid, P is proline, and C is cysteine
  SITE 16: note = Variant - X11, is present or not and, if present, is a polypeptide stretch con-sisting of the amino acid sequence LR or GSGL, wherein L is leucine, R is arginine, G is glycine, and S is serine
  SITE 17: note = Variant - X12, is present or not and, if present, is a basic polypeptide stretch with at least 20 % basic amino acid residues selected from K and R and at least a P residue, preferably wherein X12 is selected from KYKPKL, KYKPKLGT, or GX3X4X5GX6X7X8GX9X10, wherein K, R, P, L, G, T, X3, X4, X5, GX6, X7, X8, GX9, and X10, are defined as above and wherein Y is tyrosine
  SITE 18: note = Variant - X13, is present or not and, if present, is a polypeptide stretch consisting of the amino acid sequences GS, GST, GST, GSG, GSTG, or GSGL, wherein G, S, T and L are defined as above
  SITE 19: note = Variant - X14, is present or not and, if present, is an amino acid linker, wherein the polypeptide has a length from 20 to 75 amino acid residues, preferably from 24 to 65 amino acid residues, especially from 25 to 60 amino acid residues
XGXXGXXXGXXXGXXXXXX

SEQ ID NO: 2 - protein, 5 aa, synthetic construct
  REGION 1..5: note = peptide
KKKKK

SEQ ID NO: 3 - protein, 4 aa, synthetic construct
  REGION 1..4: note = peptide
KRKK

SEQ ID NO: 4 - protein, 4 aa, synthetic construct
  REGION 1..4: note = peptide
GLGS

SEQ ID NO: 5 - protein, 4 aa, synthetic construct
  REGION 1..4: note = peptide
GSGL

SEQ ID NO: 6 - protein, 6 aa, synthetic construct
  REGION 1..6: note = peptide
KYKPKL

SEQ ID NO: 7 - protein, 8 aa, synthetic construct
  REGION 1..8: note = peptide
KYKPKLGT

SEQ ID NO: 8 - skipped

SEQ ID NO: 9 - protein, 36 aa, synthetic construct
  REGION 1..36: note = peptide, DDM11
GNSGSGKRKKKGKGLGKKRDPCLRKYKPKLGTGSTG

SEQ ID NO: 10 - protein, 42 aa, synthetic construct
  REGION 1..42: note = peptide, DDM11
GNSGSGKRKKKGKGLGKKRDPCLRKYKPKLGTGSTGHHHHHH

SEQ ID NO: 11 - protein, 36 aa, synthetic construct
  REGION 1..36: note = peptide, DDM18
GNSGKRKKKGKGSGLGSGKKRDPCLRKYKPKLGSTG

SEQ ID NO: 12 - protein, 42 aa, synthetic construct
  REGION 1..42: note = peptide, DDM18
GNSGKRKKKGKGSGLGSGKKRDPCLRKYKPKLGSTGHHHHHH

SEQ ID NO: 13 - protein, 36 aa, synthetic construct; identical to SEQ ID NO: 9
  REGION 1..36: note = peptide, DDM21

SEQ ID NO: 14 - protein, 42 aa, synthetic construct; identical to SEQ ID NO: 10
  REGION 1..42: note = peptide, DDM21

SEQ ID NO: 15 - protein, 30 aa, synthetic construct
  REGION 1..30: note = peptide, DDM26
GNSGSGKRKKKGKGSGLGSGKKRDPLGSTG

SEQ ID NO: 16 - protein, 36 aa, synthetic construct
  REGION 1..36: note = peptide, DDM26
GNSGSGKRKKKGKGSGLGSGKKRDPLGSTGHHHHHH

SEQ ID NO: 17 - protein, 29 aa, synthetic construct
  REGION 1..29: note = peptide, DDM27
GNSGGSTGGKRKKKGKGSGLGSGKKRDPL

SEQ ID NO: 18 - protein, 35 aa, synthetic construct
  REGION 1..35: note = peptide, DDM27
GNSGHHHHHHGSTGGKRKKKGKGSGLGSGKKRDPL

SEQ ID NO: 19 - protein, 30 aa, synthetic construct
  REGION 1..30: note = peptide, DDM28
GNSGSGKRKKKGKGSGLGSGKKKDPLGSTG

SEQ ID NO: 20 - protein, 36 aa, synthetic construct
  REGION 1..36: note = peptide, DDM28
GNSGSGKRKKKGKGSGLGSGKKKDPLGSTGHHHHHH

SEQ ID NO: 21 - protein, 29 aa, synthetic construct
  REGION 1..29: note = peptide, DDM29
GNSGGSTGGKRKKKGKGSGLGSGKKKDPL

SEQ ID NO: 22 - protein, 35 aa, synthetic construct
  REGION 1..35: note = peptide, DDM29
GNSGHHHHHHGSTGGKRKKKGKGSGLGSGKKKDPL

SEQ ID NO: 23 - protein, 30 aa, synthetic construct
  REGION 1..30: note = peptide, DDM30
GNSGSGKKKKKGKGSGLGSGKKRDPLGSTG

SEQ ID NO: 24 - protein, 36 aa, synthetic construct
  REGION 1..36: note = peptide, DDM30
GNSGSGKKKKKGKGSGLGSGKKRDPLGSTGHHHHHH

SEQ ID NO: 25 - protein, 29 aa, synthetic construct
  REGION 1..29: note = peptide, DDM31
GNSGGSTGGKKKKKGKGSGLGSGKKRDPL

SEQ ID NO: 26 - protein, 35 aa, synthetic construct
  REGION 1..35: note = peptide, DDM31
GNSGHHHHHHGSTGGKKKKKGKGSGLGSGKKRDPL

SEQ ID NO: 27 - protein, 30 aa, synthetic construct
  REGION 1..30: note = peptide, DDM32
GNSGSGKKKKKGKGSGLGSGKKKDPLGSTG

SEQ ID NO: 28 - protein, 36 aa, synthetic construct
  REGION 1..36: note = peptide, DDM32
GNSGSGKKKKKGKGSGLGSGKKKDPLGSTGHHHHHH

SEQ ID NO: 29 - protein, 29 aa, synthetic construct
  REGION 1..29: note = peptide, DDM33
GNSGGSTGGKKKKKGKGSGLGSGKKKDPL

SEQ ID NO: 30 - protein, 35 aa, synthetic construct
  REGION 1..35: note = peptide, DDM33
GNSGHHHHHHGSTGGKKKKKGKGSGLGSGKKKDPL

SEQ ID NO: 31 - protein, 28 aa, synthetic construct
  REGION 1..28: note = peptide, DDM35
GNSGSGKKKKKGKGSGLGSGKKKLGSTG

SEQ ID NO: 32 - protein, 34 aa, synthetic construct
  REGION 1..34: note = peptide, DDM35
GNSGSGKKKKKGKGSGLGSGKKKLGSTGHHHHHH

SEQ ID NO: 33 - protein, 60 aa, synthetic construct
  REGION 1..60: note = peptide, DDM44
GNSGSGKKKKKGKGSGLGSGKKKDPLGSGLGSGKKKKKGKGSGLGSGKKKDPLGSTGGST

SEQ ID NO: 34 - protein, 26 aa, synthetic construct
  REGION 1..26: note = peptide, DDM34
GNSGSGKKKKKGKGSGLGSGKKKDPL

SEQ ID NO: 35 - protein, 66 aa, synthetic construct
  REGION 1..66: note = peptide, DDM44
GNSGSGKKKKKGKGSGLGSGKKKDPLGSGLGSGKKKKKGKGSGLGSGKKKDPLGSTGHHHHHHGST

SEQ ID NO: 36 - protein, 56 aa, synthetic construct
  REGION 1..56: note = peptide, DDM36
GNSGSGKKKKKGKGSGLGSGKKKDPLGSGLGSGKKKKKGKGSGLGSGKKKDPLGST

SEQ ID NO: 37 - protein, 156 aa, synthetic construct
  REGION 1..156: note = peptide
SHPDLNKLLELWPHIQEYQDLALKHGINDIFQDNGGKLLQVLLITGLTVLPGREGNDAVDNAGQEYELKSINIDLTKGFSTHHHMNPVIIAKYRQVPWIFAIYRGIAIEAIYRLEPKDLEFYYDKWERKWYSDGHKDINNPKIPVKYVMEHGTKIY

SEQ ID NO: 38 - protein, 160 aa, synthetic construct
  REGION 1..160: note = peptide
SHPDLNKLLELWPHIQEYQDLALKHGINDIFQDNGGKLLQVLLITGLTVLPGREGNDAVDNAGQEYELKSINIDLTKGFSTHHHMNPVIIAKYRQVPWIFAIYRGIAIEAIYRLEPKDLEFYYDKWERKWYSDGHKDINNPKIPVKYVMEHGTKIYGSGG

SEQ ID NO: 39 - protein, 160 aa, synthetic construct
  REGION 1..160: note = peptide
SGGSSHPDLNKLLELWPHIQEYQDLALKHGINDIFQDNGGKLLQVLLITGLTVLPGREGNDAVDNAGQEYELKSINIDLTKGFSTHHHMNPVIIAKYRQVPWIFAIYRGIAIEAIYRLEPKDLEFYYDKWERKWYSDGHKDINNPKIPVKYVMEHGTKIY

SEQ ID NO: 40 - protein, 160 aa, synthetic construct
  REGION 1..160: note = peptide
SHPDLNKLLELWPHIQEYQDLALKHGINDIFQDNGGKLLQVLLITGLTVLPGREGNDAVDNAGQEYELKSINIDLTKGFSTHHHMNPVIIAKYRQVPWIFAIYRGIAIEAIYRLEPKDLEFYYDKWERKWYSDGHKDINNPKIPVKYVMEHGTKIYGNSG

SEQ ID NO: 41 - protein, 157 aa, synthetic construct
  REGION 1..157: note = peptide
MSHPDLNKLLELWPHIQEYQDLALKHGINDIFQDNGGKLLQVLLITGLTVLPGREGNDAVDNAGQEYELKSINIDLTKGFSTHHHMNPVIIAKYRQVPWIFAIYRGIAIEAIYRLEPKDLEFYYDKWERKWYSDGHKDINNPKIPVKYVMEHGTKIY

SEQ ID NO: 42 - protein, 161 aa, synthetic construct
  REGION 1..161: note = peptide
SHPDLNKLLELWPHIQEYQDLALKHGINDIFQDNGGKLLQVLLITGLTVLPGREGNDAVDNAGQEYELKSINIDLTKGFSTHHHMNPVIIAKYRQVPWIFAIYRGIAIEAIYRLEPKDLEFYYDKWERKWYSDGHKDINNPKIPVKYVMEHGTKIYGSGGC

SEQ ID NO: 43 - protein, 161 aa, synthetic construct
  REGION 1..161: note = peptide
CSGGSSHPDLNKLLELWPHIQEYQDLALKHGINDIFQDNGGKLLQVLLITGLTVLPGREGNDAVDNAGQEYELKSINIDLTKGFSTHHHMNPVIIAKYRQVPWIFAIYRGIAIEAIYRLEPKDLEFYYDKWERKWYSDGHKDINNPKIPVKYVMEHGTKIY

SEQ ID NO: 44 - protein, 322 aa, synthetic construct
  REGION 1..322: note = peptide
MSHPDLNKLLELWPHIQEYQDLALKHGINDIFQDNGGKLLQVLLITGLTVLPGREGNDAVDNAGQEYELKSINIDLTKGFSTHHHMNPVIIAKYRQVPWIFAIYRGIAIEAIYRLEPKDLEFYYDKWERKWYSDGHKDINNPKIPVKYVMEHGTKIYGSGGCSGGSSHPDLNKLLELWPHIQEYQDLALKHGINDIFQDNGGKLLQVLLITGLTVLPGREGNDAVDNAGQEYELKSINIDLTKGFSTHHHMNPVIIAKYRQVPWIFAIYRGIAIEAIYRLEPKDLEFYYDKWERKWYSDGHKDINNPKIPVKYVMEHGTKIY

SEQ ID NO: 45 - protein, 321 aa, synthetic construct
  REGION 1..321: note = peptide
MSHPDLNKLLELWPHIQEYQDLALKHGINDIFQDNGGKLLQVLLITGLTVLPGREGNDAVDNAGQEYELKSINIDLTKGFSTHHHMNPVIIAKYRQVPWIFAIYRGIAIEAIYRLEPKDLEFYYDKWERKWYSDGHKDINNPKIPVKYVMEHGTKIYGSGGSGGSSHPDLNKLLELWPHIQEYQDLALKHGINDIFQDNGGKLLQVLLITGLTVLPGREGNDAVDNAGQEYELKSINIDLTKGFSTHHHMNPVIIAKYRQVPWIFAIYRGIAIEAIYRLEPKDLEFYYDKWERKWYSDGHKDINNPKIPVKYVMEHGTKIY

SEQ ID NO: 46 - protein, 165 aa, synthetic construct
  REGION 1..165: note = peptide
MSHPDLNKLLELWPHIQEYQDLALKHGINDIFQDNGGKLLQVLLITGLTVLPGREGNDAVDNAGQEYELKSINIDLTKGFSTHHHMNPVIIAKYRQVPWIFAIYRGIAIEAIYRLEPKDLEFYYDKWERKWYSDGHKDINNPKIPVKYVMEHGTKIYGSGGSGGS

SEQ ID NO: 47 - protein, 164 aa, synthetic construct
  REGION 1..164: note = peptide
SHPDLNKLLELWPHIQEYQDLALKHGINDIFQDNGGKLLQVLLITGLTVLPGREGNDAVDNAGQEYELKSINIDLTKGFSTHHHMNPVIIAKYRQVPWIFAIYRGIAIEAIYRLEPKDLEFYYDKWERKWYSDGHKDINNPKIPVKYVMEHGTKIYGSGGSGGS

SEQ ID NO: 48 - protein, 164 aa, synthetic construct
  REGION 1..164: note = peptide
GSGGSGGSSHPDLNKLLELWPHIQEYQDLALKHGINDIFQDNGGKLLQVLLITGLTVLPGREGNDAVDNAGQEYELKSINIDLTKGFSTHHHMNPVIIAKYRQVPWIFAIYRGIAIEAIYRLEPKDLEFYYDKWERKWYSDGHKDINNPKIPVKYVMEHGTKIY

SEQ ID NO: 49 - protein, 377 aa, synthetic construct
  REGION 1..377: note = peptide, CROMOC36
MSHPDLNKLLELWPHIQEYQDLALKHGINDIFQDNGGKLLQVLLITGLTVLPGREGNDAVDNAGQEYELKSINIDLTKGFSTHHHMNPVIIAKYRQVPWIFAIYRGIAIEAIYRLEPKDLEFYYDKWERKWYSDGHKDINNPKIPVKYVMEHGTKIYGSGGSGGSSHPDLNKLLELWPHIQEYQDLALKHGINDIFQDNGGKLLQVLLITGLTVLPGREGNDAVDNAGQEYELKSINIDLTKGFSTHHHMNPVIIAKYRQVPWIFAIYRGIAIEAIYRLEPKDLEFYYDKWERKWYSDGHKDINNPKIPVKYVMEHGTKIYGNSGSGKKKKKGKGSGLGSGKKKDPLGSGLGSGKKKKKGKGSGLGSGKKKDPLGST

SEQ ID NO: 50 - protein, 156 aa, synthetic construct; identical to SEQ ID NO: 37
  REGION 1..156: note = peptide

SEQ ID NO: 51 - protein, 160 aa, synthetic construct; identical to SEQ ID NO: 38
  REGION 1..160: note = peptide

SEQ ID NO: 52 - protein, 160 aa, synthetic construct; identical to SEQ ID NO: 39
  REGION 1..160: note = peptide

SEQ ID NO: 53 - protein, 160 aa, synthetic construct; identical to SEQ ID NO: 40
  REGION 1..160: note = peptide

SEQ ID NO: 54 - protein, 157 aa, synthetic construct; identical to SEQ ID NO: 41
  REGION 1..157: note = peptide

SEQ ID NO: 55 - protein, 161 aa, synthetic construct; identical to SEQ ID NO: 42
  REGION 1..161: note = peptide

SEQ ID NO: 56 - protein, 161 aa, synthetic construct; identical to SEQ ID NO: 43
  REGION 1..161: note = peptide

SEQ ID NO: 57 - protein, 322 aa, synthetic construct; identical to SEQ ID NO: 44
  REGION 1..322: note = peptide

SEQ ID NO: 58 - protein, 321 aa, synthetic construct; identical to SEQ ID NO: 45
  REGION 1..321: note = peptide

SEQ ID NO: 59 - protein, 165 aa, synthetic construct; identical to SEQ ID NO: 46
  REGION 1..165: note = peptide

SEQ ID NO: 60 - protein, 377 aa, synthetic construct
  REGION 1..377: note = peptide, CROMOC60
MSHPDLNKLLELWPHIQEYQDLALKHGINDIFQDNGGKLLQVLLITGLTVLPGREGNDAVDNAGQEYELKSINIDLTAGFSTHHHMNPVIIAKYRQVPWIFAIYRGIAIEAIYRLEPKDLEFYYDKWERKWYSDGHKDINNPKIPVKYVMEHGTKIYGSGGSGGSSHPDLNKLLELWPHIQEYQDLALKHGINDIFQDNGGKLLQVLLITGLTVLPGREGNDAVDNAGQEYELKSINIDLTAGFSTHHHMNPVIIAKYRQVPWIFAIYRGIAIEAIYRLEPKDLEFYYDKWERKWYSDGHKDINNPKIPVKYVMEHGTKIYGNSGSGKKKKKGKGSGLGSGKKKDPLGSGLGSGKKKKKGKGSGLGSGKKKDPLGST

SEQ ID NO: 61 - protein, 164 aa, synthetic construct; identical to SEQ ID NO: 47
  REGION 1..164: note = peptide

SEQ ID NO: 62 - protein, 378 aa, synthetic construct
  REGION 1..378: note = peptide, CROMOC62
MSHPDLNKLLELWPHIQEYQDLALKHGINDIFQDNGGKLLQVLLITGLTVLPGREGNDAVDNAGQEYELKSINIDLTKGFSTHHHMNPVIIAKYRQVPWIFAIYRGIAIEAIYRLEPKDLEFYYDKWERKWYSDGHKDINNPKIPVKYVMEHGTKIYGSGGCSGGSSHPDLNKLLELWPHIQEYQDLALKHGINDIFQDNGGKLLQVLLITGLTVLPGREGNDAVDNAGQEYELKSINIDLTKGFSTHHHMNPVIIAKYRQVPWIFAIYRGIAIEAIYRLEPKDLEFYYDKWERKWYSDGHKDINNPKIPVKYVMEHGTKIYGNSGSGKKKKKGKGSGLGSGKKKDPLGSGLGSGKKKKKGKGSGLGSGKKKDPLGST

SEQ ID NO: 63 - protein, 164 aa, synthetic construct; identical to SEQ ID NO: 48
  REGION 1..164: note = peptide

SEQ ID NO: 64 - protein, 4 aa, synthetic construct
  REGION 1..4: note = peptide
GSGG

SEQ ID NO: 65 - protein, 4 aa, synthetic construct
  REGION 1..4: note = peptide
SGGS

SEQ ID NO: 66 - protein, 5 aa, synthetic construct
  REGION 1..5: note = peptide
GSGGC

SEQ ID NO: 67 - protein, 5 aa, synthetic construct
  REGION 1..5: note = peptide
CSGGS

SEQ ID NO: 68 - protein, 8 aa, synthetic construct
  REGION 1..8: note = peptide
GSGGSGGS

SEQ ID NO: 69 - protein, 9 aa, synthetic construct
  REGION 1..9: note = peptide
GSGGCSGGS

SEQ ID NO: 70 - protein, 15 aa, synthetic construct
GKRKKKGKLGKKRDP

SEQ ID NO: 71 - protein, 22 aa, synthetic construct
GKRKKKGKGLGKKRDPCLRKYK

SEQ ID NO: 72 - protein, 10 aa, synthetic construct
GSGGCCSGGS

SEQ ID NO: 73 - protein, 156 aa, synthetic construct; identical to SEQ ID NO: 37

SEQ ID NO: 74 - protein, 156 aa, synthetic construct
SHPDLNKLLELWPHIQEYQDLALKHGINDIFQDNGGKLLQVLLITGLTVLPGREGNDAVDNAGQEYELASINIDLTKGFSTHHHMNPVIIAKYRQVPWIFAIYRGIAIEAIYRLEPKDLEFYYDKWERKWYSDGHKDINNPKIPVKYVMEHGTKIY

SEQ ID NO: 75 - protein, 321 aa, synthetic construct
SHPDLNKLLELWPHIQEYQDLALKHGINDIFQDNGGKLLQVLLITGLTVLPGREGNDAVDNAGQEYELKSINIDLTKGFSTHHHMNPVIIAKYRQVPWIFAIYRGIAIEAIYRLEPKDLEFYYDKWERKWYSDGHKDINNPKIPVKYVMEHGTKIYGSGGGSGGSSHPDLNKLLELWPHIQEYQDLALKHGINDIFQDNGGKLLQVLLITGLTVLPGREGNDAVDNAGQEYELKSINIDLTKGFSTHHHMNPVIIAKYRQVPWIFAIYRGIAIEAIYRLEPKDLEFYYDKWERKWYSDGHKDINNPKIPVKYVMEHGTKIY

SEQ ID NO: 76 - protein, 321 aa, synthetic construct
SHPDLNKLLELWPHIQEYQDLALKHGINDIFQDNGGKLLQVLLITGLTVLPGREGNDAVDNAGQEYELASINIDLTKGFSTHHHMNPVIIAKYRQVPWIFAIYRGIAIEAIYRLEPKDLEFYYDKWERKWYSDGHKDINNPKIPVKYVMEHGTKIYGSGGGSGGSSHPDLNKLLELWPHIQEYQDLALKHGINDIFQDNGGKLLQVLLITGLTVLPGREGNDAVDNAGQEYELASINIDLTKGFSTHHHMNPVIIAKYRQVPWIFAIYRGIAIEAIYRLEPKDLEFYYDKWERKWYSDGHKDINNPKIPVKYVMEHGTKIY

SEQ ID NO: 77 - protein, 321 aa, synthetic construct
SHPDLNKLLELWPHIQEYQDLALKHGINDIFQDNGGKLLQVLLITGLTVLPGREGNDAVDNAGQEYELKSINIDLTKGFSTHHHMNPVIIAKYRQVPWIFAIYRGIAIEAIYRLEPKDLEFYYDKWERKWYSDGHKDINNPKIPVKYVMEHGTKIYGSGGCSGGSSHPDLNKLLELWPHIQEYQDLALKHGINDIFQDNGGKLLQVLLITGLTVLPGREGNDAVDNAGQEYELKSINIDLTKGFSTHHHMNPVIIAKYRQVPWIFAIYRGIAIEAIYRLEPKDLEFYYDKWERKWYSDGHKDINNPKIPVKYVMEHGTKIY

SEQ ID NO: 78 - protein, 322 aa, synthetic construct
SHPDLNKLLELWPHIQEYQDLALKHGINDIFQDNGGKLLQVLLITGLTVLPGREGNDAVDNAGQEYELKSINIDLTKGFSTHHHMNPVIIAKYRQVPWIFAIYRGIAIEAIYRLEPKDLEFYYDKWERKWYSDGHKDINNPKIPVKYVMEHGTKIYGSGGCCSGGSSHPDLNKLLELWPHIQEYQDLALKHGINDIFQDNGGKLLQVLLITGLTVLPGREGNDAVDNAGQEYELKSINIDLTKGFSTHHHMNPVIIAKYRQVPWIFAIYRGIAIEAIYRLEPKDLEFYYDKWERKWYSDGHKDINNPKIPVKYVMEHGTKIY

SEQ ID NO: 79 - protein, 321 aa, synthetic construct
SHPDLNKLLELWPHIQEYQDLALKHGINDIFQDNGGKLLQVLLITGLTVLPGREGNDAVDNAGQEYELASINIDLTKGFSTHHHMNPVIIAKYRQVPWIFAIYRGIAIEAIYRLEPKDLEFYYDKWERKWYSDGHKDINNPKIPVKYVMEHGTKIYGSGGCSGGSSHPDLNKLLELWPHIQEYQDLALKHGINDIFQDNGGKLLQVLLITGLTVLPGREGNDAVDNAGQEYELASINIDLTKGFSTHHHMNPVIIAKYRQVPWIFAIYRGIAIEAIYRLEPKDLEFYYDKWERKWYSDGHKDINNPKIPVKYVMEHGTKIY

SEQ ID NO: 80 - protein, 322 aa, synthetic construct
SHPDLNKLLELWPHIQEYQDLALKHGINDIFQDNGGKLLQVLLITGLTVLPGREGNDAVDNAGQEYELASINIDLTKGFSTHHHMNPVIIAKYRQVPWIFAIYRGIAIEAIYRLEPKDLEFYYDKWERKWYSDGHKDINNPKIPVKYVMEHGTKIYGSGGCCSGGSSHPDLNKLLELWPHIQEYQDLALKHGINDIFQDNGGKLLQVLLITGLTVLPGREGNDAVDNAGQEYELASINIDLTKGFSTHHHMNPVIIAKYRQVPWIFAIYRGIAIEAIYRLEPKDLEFYYDKWERKWYSDGHKDINNPKIPVKYVMEHGTKIY

SEQ ID NO: 81 - protein, 323 aa, synthetic construct
SHPDLNKLLELWPHIQEYQDLALKHGINDIFQDNGGKLLQVLLITGLTVLPGREGNDAVDNAGQEYELKSINIDLTKGFSTHHHMNPVIIAKYRQVPWIFAIYRGIAIEAIYRLEPKDLEFYYDKWERKWYSDGHKDINNPKIPVKYVMEHGTKIYGSGGCCCSGGSSHPDLNKLLELWPHIQEYQDLALKHGINDIFQDNGGKLLQVLLITGLTVLPGREGNDAVDNAGQEYELKSINIDLTKGFSTHHHMNPVIIAKYRQVPWIFAIYRGIAIEAIYRLEPKDLEFYYDKWERKWYSDGHKDINNPKIPVKYVMEHGTKIY

SEQ ID NO: 82 - protein, 323 aa, synthetic construct
SHPDLNKLLELWPHIQEYQDLALKHGINDIFQDNGGKLLQVLLITGLTVLPGREGNDAVDNAGQEYELASINIDLTKGFSTHHHMNPVIIAKYRQVPWIFAIYRGIAIEAIYRLEPKDLEFYYDKWERKWYSDGHKDINNPKIPVKYVMEHGTKIYGSGGCCCSGGSSHPDLNKLLELWPHIQEYQDLALKHGINDIFQDNGGKLLQVLLITGLTVLPGREGNDAVDNAGQEYELASINIDLTKGFSTHHHMNPVIIAKYRQVPWIFAIYRGIAIEAIYRLEPKDLEFYYDKWERKWYSDGHKDINNPKIPVKYVMEHGTKIY

SEQ ID NO: 83 - protein, 212 aa, synthetic construct
SHPDLNKLLELWPHIQEYQDLALKHGINDIFQDNGGKLLQVLLITGLTVLPGREGNDAVDNAGQEYELKSINIDLTKGFSTHHHMNPVIIAKYRQVPWIFAIYRGIAIEAIYRLEPKDLEFYYDKWERKWYSDGHKDINNPKIPVKYVMEHGTKIYGNSGSGKKKKKGKGSGLGSGKKKDPLGSGLGSGKKKKKGKGSGLGSGKKKDPLGST

SEQ ID NO: 84 - protein, 212 aa, synthetic construct
SHPDLNKLLELWPHIQEYQDLALKHGINDIFQDNGGKLLQVLLITGLTVLPGREGNDAVDNAGQEYELASINIDLTKGFSTHHHMNPVIIAKYRQVPWIFAIYRGIAIEAIYRLEPKDLEFYYDKWERKWYSDGHKDINNPKIPVKYVMEHGTKIYGNSGSGKKKKKGKGSGLGSGKKKDPLGSGLGSGKKKKKGKGSGLGSGKKKDPLGST

SEQ ID NO: 85 - protein, 377 aa, synthetic construct
SHPDLNKLLELWPHIQEYQDLALKHGINDIFQDNGGKLLQVLLITGLTVLPGREGNDAVDNAGQEYELKSINIDLTKGFSTHHHMNPVIIAKYRQVPWIFAIYRGIAIEAIYRLEPKDLEFYYDKWERKWYSDGHKDINNPKIPVKYVMEHGTKIYGSGGGSGGSSHPDLNKLLELWPHIQEYQDLALKHGINDIFQDNGGKLLQVLLITGLTVLPGREGNDAVDNAGQEYELKSINIDLTKGFSTHHHMNPVIIAKYRQVPWIFAIYRGIAIEAIYRLEPKDLEFYYDKWERKWYSDGHKDINNPKIPVKYVMEHGTKIYGNSGSGKKKKKGKGSGLGSGKKKDPLGSGLGSGKKKKKGKGSGLGSGKKKDPLGST

SEQ ID NO: 86 - protein, 377 aa, synthetic construct
SHPDLNKLLELWPHIQEYQDLALKHGINDIFQDNGGKLLQVLLITGLTVLPGREGNDAVDNAGQEYELASINIDLTKGFSTHHHMNPVIIAKYRQVPWIFAIYRGIAIEAIYRLEPKDLEFYYDKWERKWYSDGHKDINNPKIPVKYVMEHGTKIYGSGGGSGGSSHPDLNKLLELWPHIQEYQDLALKHGINDIFQDNGGKLLQVLLITGLTVLPGREGNDAVDNAGQEYELASINIDLTKGFSTHHHMNPVIIAKYRQVPWIFAIYRGIAIEAIYRLEPKDLEFYYDKWERKWYSDGHKDINNPKIPVKYVMEHGTKIYGNSGSGKKKKKGKGSGLGSGKKKDPLGSGLGSGKKKKKGKGSGLGSGKKKDPLGST

SEQ ID NO: 87 - protein, 377 aa, synthetic construct
SHPDLNKLLELWPHIQEYQDLALKHGINDIFQDNGGKLLQVLLITGLTVLPGREGNDAVDNAGQEYELKSINIDLTKGFSTHHHMNPVIIAKYRQVPWIFAIYRGIAIEAIYRLEPKDLEFYYDKWERKWYSDGHKDINNPKIPVKYVMEHGTKIYGSGGCSGGSSHPDLNKLLELWPHIQEYQDLALKHGINDIFQDNGGKLLQVLLITGLTVLPGREGNDAVDNAGQEYELKSINIDLTKGFSTHHHMNPVIIAKYRQVPWIFAIYRGIAIEAIYRLEPKDLEFYYDKWERKWYSDGHKDINNPKIPVKYVMEHGTKIYGNSGSGKKKKKGKGSGLGSGKKKDPLGSGLGSGKKKKKGKGSGLGSGKKKDPLGST

SEQ ID NO: 88 - protein, 378 aa, synthetic construct
SHPDLNKLLELWPHIQEYQDLALKHGINDIFQDNGGKLLQVLLITGLTVLPGREGNDAVDNAGQEYELKSINIDLTKGFSTHHHMNPVIIAKYRQVPWIFAIYRGIAIEAIYRLEPKDLEFYYDKWERKWYSDGHKDINNPKIPVKYVMEHGTKIYGSGGCCSGGSSHPDLNKLLELWPHIQEYQDLALKHGINDIFQDNGGKLLQVLLITGLTVLPGREGNDAVDNAGQEYELKSINIDLTKGFSTHHHMNPVIIAKYRQVPWIFAIYRGIAIEAIYRLEPKDLEFYYDKWERKWYSDGHKDINNPKIPVKYVMEHGTKIYGNSGSGKKKKKGKGSGLGSGKKKDPLGSGLGSGKKKKKGKGSGLGSGKKKDPLGST

SEQ ID NO: 89 - protein, 377 aa, synthetic construct
SHPDLNKLLELWPHIQEYQDLALKHGINDIFQDNGGKLLQVLLITGLTVLPGREGNDAVDNAGQEYELASINIDLTKGFSTHHHMNPVIIAKYRQVPWIFAIYRGIAIEAIYRLEPKDLEFYYDKWERKWYSDGHKDINNPKIPVKYVMEHGTKIYGSGGCSGGSSHPDLNKLLELWPHIQEYQDLALKHGINDIFQDNGGKLLQVLLITGLTVLPGREGNDAVDNAGQEYELASINIDLTKGFSTHHHMNPVIIAKYRQVPWIFAIYRGIAIEAIYRLEPKDLEFYYDKWERKWYSDGHKDINNPKIPVKYVMEHGTKIYGNSGSGKKKKKGKGSGLGSGKKKDPLGSGLGSGKKKKKGKGSGLGSGKKKDPLGST

SEQ ID NO: 90 - protein, 378 aa, synthetic construct
SHPDLNKLLELWPHIQEYQDLALKHGINDIFQDNGGKLLQVLLITGLTVLPGREGNDAVDNAGQEYELASINIDLTKGFSTHHHMNPVIIAKYRQVPWIFAIYRGIAIEAIYRLEPKDLEFYYDKWERKWYSDGHKDINNPKIPVKYVMEHGTKIYGSGGCCSGGSSHPDLNKLLELWPHIQEYQDLALKHGINDIFQDNGGKLLQVLLITGLTVLPGREGNDAVDNAGQEYELASINIDLTKGFSTHHHMNPVIIAKYRQVPWIFAIYRGIAIEAIYRLEPKDLEFYYDKWERKWYSDGHKDINNPKIPVKYVMEHGTKIYGNSGSGKKKKKGKGSGLGSGKKKDPLGSGLGSGKKKKKGKGSGLGSGKKKDPLGST

SEQ ID NO: 91 - protein, 379 aa, synthetic construct
SHPDLNKLLELWPHIQEYQDLALKHGINDIFQDNGGKLLQVLLITGLTVLPGREGNDAVDNAGQEYELKSINIDLTKGFSTHHHMNPVIIAKYRQVPWIFAIYRGIAIEAIYRLEPKDLEFYYDKWERKWYSDGHKDINNPKIPVKYVMEHGTKIYGSGGCCCSGGSSHPDLNKLLELWPHIQEYQDLALKHGINDIFQDNGGKLLQVLLITGLTVLPGREGNDAVDNAGQEYELKSINIDLTKGFSTHHHMNPVIIAKYRQVPWIFAIYRGIAIEAIYRLEPKDLEFYYDKWERKWYSDGHKDINNPKIPVKYVMEHGTKIYGNSGSGKKKKKGKGSGLGSGKKKDPLGSGLGSGKKKKKGKGSGLGSGKKKDPLGST

SEQ ID NO: 92 - protein, 379 aa, synthetic construct
SHPDLNKLLELWPHIQEYQDLALKHGINDIFQDNGGKLLQVLLITGLTVLPGREGNDAVDNAGQEYELASINIDLTKGFSTHHHMNPVIIAKYRQVPWIFAIYRGIAIEAIYRLEPKDLEFYYDKWERKWYSDGHKDINNPKIPVKYVMEHGTKIYGSGGCCCSGGSSHPDLNKLLELWPHIQEYQDLALKHGINDIFQDNGGKLLQVLLITGLTVLPGREGNDAVDNAGQEYELASINIDLTKGFSTHHHMNPVIIAKYRQVPWIFAIYRGIAIEAIYRLEPKDLEFYYDKWERKWYSDGHKDINNPKIPVKYVMEHGTKIYGNSGSGKKKKKGKGSGLGSGKKKDPLGSGLGSGKKKKKGKGSGLGSGKKKDPLGST

SEQ ID NO: 93 - protein, 11 aa, synthetic construct
GSGGCCCSGGS

SEQ ID NO: 94 - protein, 380 aa, synthetic construct
SHPDLNKLLELWPHIQEYQDLALKHGINDIFQDNGGKLLQVLLITGLTVLPGREGNDAVDNAGQEYELKSINIDLTKGFSTHHHMNPVIIAKYRQVPWIFAIYRGIAIEAIYRLEPKDLEFYYDKWERKWYSDGHKDINNPKIPVKYVMEHGTKIYGSGGCAACSGGSSHPDLNKLLELWPHIQEYQDLALKHGINDIFQDNGGKLLQVLLITGLTVLPGREGNDAVDNAGQEYELKSINIDLTKGFSTHHHMNPVIIAKYRQVPWIFAIYRGIAIEAIYRLEPKDLEFYYDKWERKWYSDGHKDINNPKIPVKYVMEHGTKIYGNSGSGKKKKKGKGSGLGSGKKKDPLGSGLGSGKKKKKGKGSGLGSGKKKDPLGST

SEQ ID NO: 95 - protein, 381 aa, synthetic construct
SHPDLNKLLELWPHIQEYQDLALKHGINDIFQDNGGKLLQVLLITGLTVLPGREGNDAVDNAGQEYELKSINIDLTKGFSTHHHMNPVIIAKYRQVPWIFAIYRGIAIEAIYRLEPKDLEFYYDKWERKWYSDGHKDINNPKIPVKYVMEHGTKIYGSGCAACAACSGSSHPDLNKLLELWPHIQEYQDLALKHGINDIFQDNGGKLLQVLLITGLTVLPGREGNDAVDNAGQEYELKSINIDLTKGFSTHHHMNPVIIAKYRQVPWIFAIYRGIAIEAIYRLEPKDLEFYYDKWERKWYSDGHKDINNPKIPVKYVMEHGTKIYGNSGSGKKKKKGKGSGLGSGKKKDPLGSGLGSGKKKKKGKGSGLGSGKKKDPLGST